European Patent Application EP 4 209 500 A1, published July 12, 2023. Title: PEPTIDE AND COMPOSITION FOR IMPROVING WRINKLE AND TREATING METABOLIC DESEASE CONTAINING THE SAME. Applicant: SEOUL NATIONAL UNIVERSITY HOSPITAL. The sequence listing filed with the application follows.

SEQUENCE LISTING (2 sequences)

SEQ ID NO: 1 - protein, 4 aa, Artificial Sequence
  Adiponectin derived peptide
LYYF

SEQ ID NO: 2 - protein, 5 aa, Artificial Sequence
  Adiponectin derived peptide
GLYYF